European Patent Specification EP 3 459 974 B1, published February 19, 2025. Title: SPECIFIC PLASMIN INACTIVATION BY ANTICATALYTIC ANTIBODY. Applicant: TRANSLATIONAL SCIENCES, INC. The sequence listing filed with the application follows.

SEQUENCE LISTING (16 sequences)

SEQ ID NO: 1 - protein, 213 aa, Artificial Sequence
  Description of Artificial Sequence: Synthetic polypeptide
DIQMTQSPSSLSASLGGKVSITCKASQDINKYISWYQHKPGKGPRLLIHYTSTLQPGIPSRFSGSGSGRDYSFSISNLEPEDIATYYCLQYDNLYTFGGGTKLEIKRADAAPTVSIFPPSSEQLTSGGASVVCFLNNFYPKDINVKWKIDGSERQNGVLNSWTDQDSKDSTYSMSSTLTLTKDEYERHNSYTCEATHKTSTSPIVKSFNWNEC

SEQ ID NO: 2 - DNA, 639 bp, Artificial Sequence
  Description of Artificial Sequence: Synthetic polynucleotide
  CDS (1)..(639)
gacatccagatgacacagtctccatcctcactgtctgcatctctggggggcaaagtctccatcacttgcaaggcaagccaagacattaacaagtatatttcttggtaccaacacaagcctggaaaaggtcctaggctgctcatacattacacatctacattacagccaggcatcccatcaaggttcagtggaagtgggtctgggagagattattccttcagcatcagcaacctggagcctgaagatattgcaacttattattgtctacagtatgataatctgtacacgttcggaggggggaccaagctggaaataaaacgggcagatgctgcaccaactgtatccatcttcccaccatccagtgagcagttaacatctggaggtgcctcagtcgtgtgcttcttgaacaacttctaccccaaagacatcaatgtcaagtggaagattgatggcagtgaacgacaaaatggcgtcctgaacagttggactgatcaggacagcaaagacagcacctacagcatgagcagcaccctcacgttgaccaaggacgaatatgaacgacataacagctatacctgtgaggccactcacaagacatcaacttcacccattgtcaagagcttcaactggaatgagtgt

SEQ ID NO: 3 - DNA, 639 bp, Artificial Sequence
  Description of Artificial Sequence: Synthetic polynucleotide
acactcattccagttgaagctcttgacaatgggtgaagttgatgtcttgtgagtggcctcacaggtatagctgttatgtcgttcatattcgtccttggtcaacgtgagggtgctgctcatgctgtaggtgctgtctttgctgtcctgatcagtccaactgttcaggacgccattttgtcgttcactgccatcaatcttccacttgacattgatgtctttggggtagaagttgttcaagaagcacacgactgaggcacctccagatgttaactgctcactggatggtgggaagatggatacagttggtgcagcatctgcccgttttatttccagcttggtcccccctccgaacgtgtacagattatcatactgtagacaataataagttgcaatatcttcaggctccaggttgctgatgctgaaggaataatctctcccagacccacttccactgaaccttgatgggatgcctggctgtaatgtagatgtgtaatgtatgagcagcctaggaccttttccaggcttgtgttggtaccaagaaatatacttgttaatgtcttggcttgccttgcaagtgatggagactttgccccccagagatgcagacagtgaggatggagactgtgtcatctggatgtc

SEQ ID NO: 4 - protein, 444 aa, Artificial Sequence
  Description of Artificial Sequence: Synthetic polypeptide
EVKLLESGGGLVQPGGSLKLSCAASGFDFSRYWMSWVRQAPGKGLEWIGEINPDSSTINYTPSLKDKFIISRDNAKNSLYLQMSKVRSEDTALYYCASYCGYSYDALDCWGQGTSVTVSSAKTTPPSVYPLAPGSAAQTNSMVTLGCLVKGYFPEPVTVTWNSGSLSSGVHTFPAVLQSDLYTLSSSVTVPSSTWPSETVTCNVAHPASSTKVDKKIVPRDCGCKPCICTVPEVSSVFIFPPKPKDVLTITLTPKVTCVVVDISKDDPEVQFSWFVDDVEVHTAQTQPREEQFNSTFRSVSELPIMHQDWLNGKEFKCRVNSVAFPAPIEKTISKTKGRPKAPQVYTIPPPKEQMAKDKVSLTCMITDFFPEDITVEWQWNGQPAENYKNTQPIMDTDGSYFVYGKLNVQKSNWEAGNTFTCSVLHEGLHNHHTEKSLSHSPGK

SEQ ID NO: 5 - DNA, 1332 bp, Artificial Sequence
  Description of Artificial Sequence: Synthetic polynucleotide
  CDS (1)..(1332)
gaggtgaagcttctcgagtctggaggtggcctggtgcagcctggaggatccctgaaactctcctgtgcagcctcaggattcgattttagtagatactggatgagttgggtccggcaggctccagggaaagggctagaatggattggagaaattaatccagatagcagtacgataaactatacgccatctctaaaggataagttcatcatctccagagacaacgccaaaaattcgctgtacctgcaaatgagcaaagtgagatctgaggacacagccctttattactgtgcaagttactgcggttatagctacgatgctctggactgctggggtcaaggaacctcagtcaccgtctcctcagccaaaacgacacccccatctgtctatccactggcccctggatctgctgcccaaactaactccatggtgaccctgggatgcctggtcaagggctatttccctgagccagtgacagtgacctggaactctggatccctgtccagcggtgtgcacaccttcccagctgtcctgcagtctgacctctacactctgagcagctcagtgactgtcccctccagcacctggcccagcgagaccgtcacctgcaacgttgcccacccggccagcagcaccaaggtggacaagaaaattgtgcccagggattgtggttgtaagccttgcatatgtacagtcccagaagtatcatctgtcttcatcttccccccaaagcccaaggatgtgctcaccattactctgactcctaaggtcacgtgtgttgtggtagacatcagcaaggatgatcccgaggtccagttcagctggtttgtagatgatgtggaggtgcacacagctcagacgcaaccccgggaggagcagttcaacagcactttccgctcagtcagtgaacttcccatcatgcaccaggactggctcaatggcaaggagttcaaatgcagggtcaacagtgtagctttccctgcccccatcgagaaaaccatctccaaaaccaaaggcagaccgaaggctccacaggtgtacaccattccacctcccaaggagcagatggccaaggataaagtcagtctgacctgcatgataacagacttcttccctgaagacattactgtggagtggcagtggaatgggcagccagcggagaactacaagaacactcagcccatcatggacacagatggctcttacttcgtctacggcaagctcaatgtgcagaagagcaactgggaggcaggaaatactttcacctgctctgtgttacatgagggcctgcacaaccaccatactgagaagagcctctcccactctcctggtaaa

SEQ ID NO: 6 - DNA, 1332 bp, Artificial Sequence
  Description of Artificial Sequence: Synthetic polynucleotide
tttaccaggagagtgggagaggctcttctcagtatggtggttgtgcaggccctcatgtaacacagagcaggtgaaagtatttcctgcctcccagttgctcttctgcacattgagcttgccgtagacgaagtaagagccatctgtgtccatgatgggctgagtgttcttgtagttctccgctggctgcccattccactgccactccacagtaatgtcttcagggaagaagtctgttatcatgcaggtcagactgactttatccttggccatctgctccttgggaggtggaatggtgtacacctgtggagccttcggtctgcctttggttttggagatggttttctcgatgggggcagggaaagctacactgttgaccctgcatttgaactccttgccattgagccagtcctggtgcatgatgggaagttcactgactgagcggaaagtgctgttgaactgctcctcccggggttgcgtctgagctgtgtgcacctccacatcatctacaaaccagctgaactggacctcgggatcatccttgctgatgtctaccacaacacacgtgaccttaggagtcagagtaatggtgagcacatccttgggctttggggggaagatgaagacagatgatacttctgggactgtacatatgcaaggcttacaaccacaatccctgggcacaattttcttgtccaccttggtgctgctggccgggtgggcaacgttgcaggtgacggtctcgctgggccaggtgctggaggggacagtcactgagctgctcagagtgtagaggtcagactgcaggacagctgggaaggtgtgcacaccgctggacagggatccagagttccaggtcactgtcactggctcagggaaatagcccttgaccaggcatcccagggtcaccatggagttagtttgggcagcagatccaggggccagtggatagacagatgggggtgtcgttttggctgaggagacggtgactgaggttccttgaccccagcagtccagagcatcgtagctataaccgcagtaacttgcacagtaataaagggctgtgtcctcagatctcactttgctcatttgcaggtacagcgaatttttggcgttgtctctggagatgatgaacttatcctttagagatggcgtatagtttatcgtactgctatctggattaatttctccaatccattctagccctttccctggagcctgccggacccaactcatccagtatctactaaaatcgaatcctgaggctgcacaggagagtttcagggatcctccaggctgcaccaggccacctccagactcgagaagcttcacctc

SEQ ID NO: 7 - protein, 233 aa, Artificial Sequence
  Description of Artificial Sequence: Synthetic polypeptide
MYRMQLLSCIALSLALVTNSDIQMTQSPSSLSASLGGKVSITCKASQDINKYISWYQHKPGKGPRLLIHYTSTLQPGIPSRFSGSGSGRDYSFSISNLEPEDIATYYCLQYDNLYTFGGGTKLEIKRTVAAPSVFIFPPSDEQLKSGTASVVCLLNNFYPREAKVQWKVDNALQSGNSQESVTEQDSKDSTYSLSSTLTLSKADYEKHKVYACEVTHQGLSSPVTKSFNRGEC

SEQ ID NO: 8 - protein, 253 aa, Artificial Sequence
  Description of Artificial Sequence: Synthetic polypeptide
MYRMQLLSCIALSLALVTNSEVKLLESGGGLVQPGGSLKLSCAASGFDFSRYWMSWVRQAPGKGLEWIGEINPDSSTINYTPSLKDKFIISRDNAKNSLYLQMSKVRSEDTALYYCASYCGYSYDALDCWGQGTSVTVSSASTKGPSVFPLAPSSKSTSGGTAALGCLVKDYFPEPVTVSWNSGALTSGVHTFPAVLQSSGLYSLSSVVTVPSSSLGTQTYICNVNHKPSNTKVDKKVEPKSCDKTHTCPPCP

SEQ ID NO: 9 - protein, 6 aa, Artificial Sequence
  Description of Artificial Sequence: Synthetic peptide
QDINKY

SEQ ID NO: 10 - protein, 3 aa, Artificial Sequence
  Description of Artificial Sequence: Synthetic peptide
YTS

SEQ ID NO: 11 - protein, 8 aa, Artificial Sequence
  Description of Artificial Sequence: Synthetic peptide
LQYDNLYT

SEQ ID NO: 12 - protein, 8 aa, Artificial Sequence
  Description of Artificial Sequence: Synthetic peptide
GFDFSRYW

SEQ ID NO: 13 - protein, 8 aa, Artificial Sequence
  Description of Artificial Sequence: Synthetic peptide
INPDSSTI

SEQ ID NO: 14 - protein, 13 aa, Artificial Sequence
  Description of Artificial Sequence: Synthetic peptide
ASYCGYSYDALDC

SEQ ID NO: 15 - protein, 106 aa, Artificial Sequence
  Description of Artificial Sequence: Synthetic polypeptide
DIQMTQSPSSLSASLGGKVSITCKASQDINKYISWYQHKPGKGPRLLIHYTSTLQPGIPSRFSGSGSGRDYSFSISNLEPEDIATYYCLQYDNLYTFGGGTKLEIK

SEQ ID NO: 16 - protein, 120 aa, Artificial Sequence
  Description of Artificial Sequence: Synthetic polypeptide
EVKLLESGGGLVQPGGSLKLSCAASGFDFSRYWMSWVRQAPGKGLEWIGEINPDSSTINYTPSLKDKFIISRDNAKNSLYLQMSKVRSEDTALYYCASYCGYSYDALDCWGQGTSVTVSS